European Patent Specification EP 4 175 968 B1, published July 3, 2024. Title: METHODS AND COMPOSITIONS FOR PROTEIN SYNTHESIS AND SECRETION. Applicant: Helaina Inc. The sequence listing filed with the application follows.

SEQUENCE LISTING (49 sequences)

SEQ ID NO: 1 - protein, 90 aa, synthetic construct
MKFISILFLLIGSVFGAPVNTTTEDETAQIPAEAVIGYSDLEGDFDVAVLPFSNSTNNGLLFINTTIASIAAKEEGVSLEKREAEAYVEF

SEQ ID NO: 2 - protein, 93 aa, synthetic construct
MQFGKVLFAISALAVTALGAPVNTTTEDETAQIPAEAVIGYSDLEGDFDVAVLPFSNSTNNGLLFINTTIASIAAKEEGVSLEKREAEAYVEF

SEQ ID NO: 3 - protein, 32 aa, synthetic construct
MKFISILFLLIGSVFGAPVAPAEEAANHLHKR

SEQ ID NO: 4 - protein, 35 aa, synthetic construct
MQFGKVLFAISALAVTALGAPVAPAEEAANHLHKR

SEQ ID NO: 5 - protein, 781 aa, synthetic construct
MKFISILFLLIGSVFGAPVNTTTEDETAQIPAEAVIGYSDLEGDFDVAVLPFSNSTNNGLLFINTTIASIAAKEEGVSLEKREAEAYVEFGRRRSVQWCAVSQPEATKCFQWQRNMRKVRGPPVSCIKRDSPIQCIQAIAENRADAVTLDGGFIYEAGLAPYKLRPVAAEVYGTERQPRTHYYAVAVVKKGGSFQLNELQGLKSCHTGLRRTAGWNVPIGTLRPFLNWTGPPEPIEAAVARFFSASCVPGADKGQFPNLCRLCAGTGENKCAFSSQEPYFSYSGAFKCLRDGAGDVAFIRESTVFEDLSDEAERDEYELLCPDNTRKPVDKFKDCHLARVPSHAVVARSVNGKEDAIWNLLRQAQEKFGKDKSPKFQLFGSPSGQKDLLFKDSAIGFSRVPPRIDSGLYLGSGYFTAIQNLRKSEEEVAARRARVVWCAVGEQELRKCNQWSGLSEGSVTCSSASTTEDCIALVLKGEADAMSLDGGYVYTAGKCGLVPVLAENYKSQQSSDPDPNCVDRPVEGYLAVAVVRRSDTSLTWNSVKGKKSCHTAVDRTAGWNIPMGLLFNQTGSCKFDEYFSQSCAPGSDPRSNLCALCIGDEQGENKCVPNSNERYYGYTGAFRCLAENAGDVAFVKDVTVLQNTDGNNNEAWAKDLKLADFALLCLDGKRKPVTEARSCHLAMAPNHAVVSRMDKVERLKQVLLHQQAKFGRNGSDCPDKFCLFQSETKNLLFNDNTECLARLHGKTTYEKYLGPQYVAGITNLKKCSTSPLLEACEFLRK

SEQ ID NO: 6 - protein, 784 aa, synthetic construct
MQFGKVLFAISALAVTALGAPVNTTTEDETAQIPAEAVIGYSDLEGDFDVAVLPFSNSTNNGLLFINTTIASIAAKEEGVSLEKREAEAYVEFGRRRSVQWCAVSQPEATKCFQWQRNMRKVRGPPVSCIKRDSPIQCIQAIAENRADAVTLDGGFIYEAGLAPYKLRPVAAEVYGTERQPRTHYYAVAVVKKGGSFQLNELQGLKSCHTGLRRTAGWNVPIGTLRPFLNWTGPPEPIEAAVARFFSASCVPGADKGQFPNLCRLCAGTGENKCAFSSQEPYFSYSGAFKCLRDGAGDVAFIRESTVFEDLSDEAERDEYELLCPDNTRKPVDKFKDCHLARVPSHAVVARSVNGKEDAIWNLLRQAQEKFGKDKSPKFQLFGSPSGQKDLLFKDSAIGFSRVPPRIDSGLYLGSGYFTAIQNLRKSEEEVAARRARVVWCAVGEQELRKCNQWSGLSEGSVTCSSASTTEDCIALVLKGEADAMSLDGGYVYTAGKCGLVPVLAENYKSQQSSDPDPNCVDRPVEGYLAVAVVRRSDTSLTWNSVKGKKSCHTAVDRTAGWNIPMGLLFNQTGSCKFDEYFSQSCAPGSDPRSNLCALCIGDEQGENKCVPNSNERYYGYTGAFRCLAENAGDVAFVKDVTVLQNTDGNNNEAWAKDLKLADFALLCLDGKRKPVTEARSCHLAMAPNHAVVSRMDKVERLKQVLLHQQAKFGRNGSDCPDKFCLFQSETKNLLFNDNTECLARLHGKTTYEKYLGPQYVAGITNLKKCSTSPLLEACEFLRK

SEQ ID NO: 7 - protein, 723 aa, synthetic construct
MKFISILFLLIGSVFGAPVAPAEEAANHLHKRGRRRSVQWCAVSQPEATKCFQWQRNMRKVRGPPVSCIKRDSPIQCIQAIAENRADAVTLDGGFIYEAGLAPYKLRPVAAEVYGTERQPRTHYYAVAVVKKGGSFQLNELQGLKSCHTGLRRTAGWNVPIGTLRPFLNWTGPPEPIEAAVARFFSASCVPGADKGQFPNLCRLCAGTGENKCAFSSQEPYFSYSGAFKCLRDGAGDVAFIRESTVFEDLSDEAERDEYELLCPDNTRKPVDKFKDCHLARVPSHAVVARSVNGKEDAIWNLLRQAQEKFGKDKSPKFQLFGSPSGQKDLLFKDSAIGFSRVPPRIDSGLYLGSGYFTAIQNLRKSEEEVAARRARVVWCAVGEQELRKCNQWSGLSEGSVTCSSASTTEDCIALVLKGEADAMSLDGGYVYTAGKCGLVPVLAENYKSQQSSDPDPNCVDRPVEGYLAVAVVRRSDTSLTWNSVKGKKSCHTAVDRTAGWNIPMGLLFNQTGSCKFDEYFSQSCAPGSDPRSNLCALCIGDEQGENKCVPNSNERYYGYTGAFRCLAENAGDVAFVKDVTVLQNTDGNNNEAWAKDLKLADFALLCLDGKRKPVTEARSCHLAMAPNHAVVSRMDKVERLKQVLLHQQAKFGRNGSDCPDKFCLFQSETKNLLFNDNTECLARLHGKTTYEKYLGPQYVAGITNLKKCSTSPLLEACEFLRK

SEQ ID NO: 8 - protein, 726 aa, synthetic construct
MQFGKVLFAISALAVTALGAPVAPAEEAANHLHKRGRRRSVQWCAVSQPEATKCFQWQRNMRKVRGPPVSCIKRDSPIQCIQAIAENRADAVTLDGGFIYEAGLAPYKLRPVAAEVYGTERQPRTHYYAVAVVKKGGSFQLNELQGLKSCHTGLRRTAGWNVPIGTLRPFLNWTGPPEPIEAAVARFFSASCVPGADKGQFPNLCRLCAGTGENKCAFSSQEPYFSYSGAFKCLRDGAGDVAFIRESTVFEDLSDEAERDEYELLCPDNTRKPVDKFKDCHLARVPSHAVVARSVNGKEDAIWNLLRQAQEKFGKDKSPKFQLFGSPSGQKDLLFKDSAIGFSRVPPRIDSGLYLGSGYFTAIQNLRKSEEEVAARRARVVWCAVGEQELRKCNQWSGLSEGSVTCSSASTTEDCIALVLKGEADAMSLDGGYVYTAGKCGLVPVLAENYKSQQSSDPDPNCVDRPVEGYLAVAVVRRSDTSLTWNSVKGKKSCHTAVDRTAGWNIPMGLLFNQTGSCKFDEYFSQSCAPGSDPRSNLCALCIGDEQGENKCVPNSNERYYGYTGAFRCLAENAGDVAFVKDVTVLQNTDGNNNEAWAKDLKLADFALLCLDGKRKPVTEARSCHLAMAPNHAVVSRMDKVERLKQVLLHQQAKFGRNGSDCPDKFCLFQSETKNLLFNDNTECLARLHGKTTYEKYLGPQYVAGITNLKKCSTSPLLEACEFLRK

SEQ ID NO: 9 - protein, 691 aa, Homo Sapiens
GRRRSVQWCAVSQPEATKCFQWQRNMRKVRGPPVSCIKRDSPIQCIQAIAENRADAVTLDGGFIYEAGLAPYKLRPVAAEVYGTERQPRTHYYAVAVVKKGGSFQLNELQGLKSCHTGLRRTAGWNVPIGTLRPFLNWTGPPEPIEAAVARFFSASCVPGADKGQFPNLCRLCAGTGENKCAFSSQEPYFSYSGAFKCLRDGAGDVAFIRESTVFEDLSDEAERDEYELLCPDNTRKPVDKFKDCHLARVPSHAVVARSVNGKEDAIWNLLRQAQEKFGKDKSPKFQLFGSPSGQKDLLFKDSAIGFSRVPPRIDSGLYLGSGYFTAIQNLRKSEEEVAARRARVVWCAVGEQELRKCNQWSGLSEGSVTCSSASTTEDCIALVLKGEADAMSLDGGYVYTAGKCGLVPVLAENYKSQQSSDPDPNCVDRPVEGYLAVAVVRRSDTSLTWNSVKGKKSCHTAVDRTAGWNIPMGLLFNQTGSCKFDEYFSQSCAPGSDPRSNLCALCIGDEQGENKCVPNSNERYYGYTGAFRCLAENAGDVAFVKDVTVLQNTDGNNNEAWAKDLKLADFALLCLDGKRKPVTEARSCHLAMAPNHAVVSRMDKVERLKQVLLHQQAKFGRNGSDCPDKFCLFQSETKNLLFNDNTECLARLHGKTTYEKYLGPQYVAGITNLKKCSTSPLLEACEFLRK

SEQ ID NO: 10 - protein, 19 aa, Saccharomyces cerevisiae
MRFPSIFTAVLFAASSALA

SEQ ID NO: 11 - protein, 74 aa, Saccharomyces cerevisiae
APVNTTTEDETAQIPAEAVIGYSDLEGDFDVAVLPFSNSTNNGLLFINTTIASIAAKEEGVSLEKREAEAYVEF

SEQ ID NO: 12 - protein, 16 aa, Pichia pastoris
MKFISILFLLIGSVFG

SEQ ID NO: 13 - protein, 16 aa, Pichia pastoris
APVAPAEEAANHLHKR

SEQ ID NO: 14 - protein, 19 aa, Pichia pastoris
MQFGKVLFAISALAVTALG

SEQ ID NO: 15 - DNA, 320 bp, synthetic construct
  source 1..320: mol_type = other DNA
atgcagtttggaaaggttctatttgctatttctgccctggctgtcacagctctgggagctccagttgctccagccgaagaggcagcaaaccacttgcacaagcgtatgaggcaggtttggttctcttggattgtgggattgttcctatgttttttcaacgtgtcttctgctaaacgatgaaattcatctcaattctgttccttttgataggcagtgtatttggtatgaaattcatctcaattctgttccttttgataggcagtgtatttggtgctccagttgctccagccgaagaggcagcaaaccacttgcacaagcgt

SEQ ID NO: 16 - DNA, 34 bp, synthetic construct
  source 1..34: mol_type = other DNA
cgaaggatccaaacgatgaaattcatctcaattc

SEQ ID NO: 17 - DNA, 28 bp, synthetic construct
  source 1..28: mol_type = other DNA
gtagtgttgactggagcaccaaatacac

SEQ ID NO: 18 - DNA, 28 bp, synthetic construct
  source 1..28: mol_type = other DNA
ggtgctccagtcaacactacaacagaag

SEQ ID NO: 19 - DNA, 32 bp, synthetic construct
  source 1..32: mol_type = other DNA
ttcatcgtttggatccttcgaataattagttg

SEQ ID NO: 20 - DNA, 31 bp, synthetic construct
  source 1..31: mol_type = other DNA
cgaaggatccaaacgatgcagtttggaaagg

SEQ ID NO: 21 - DNA, 28 bp, synthetic construct
  source 1..28: mol_type = other DNA
tgactggagctcccagagctgtgacagc

SEQ ID NO: 22 - DNA, 30 bp, synthetic construct
  source 1..30: mol_type = other DNA
agctctgggagctccagtcaacactacaac

SEQ ID NO: 23 - DNA, 39 bp, synthetic construct
  source 1..39: mol_type = other DNA
tgcatcgtttggatccttcgaataattagttgttttttg

SEQ ID NO: 24 - DNA, 40 bp, synthetic construct
  source 1..40: mol_type = other DNA
gatccaaacgatgaaattcatctcaattctgttccttttg

SEQ ID NO: 25 - DNA, 30 bp, synthetic construct
  source 1..30: mol_type = other DNA
ttcttccggcacgcttgtgcaagtggtttg

SEQ ID NO: 26 - DNA, 29 bp, synthetic construct
  source 1..29: mol_type = other DNA
gcacaagcgtgccggaagaagaagaagtg

SEQ ID NO: 27 - DNA, 34 bp, synthetic construct
  source 1..34: mol_type = other DNA
tgaatttcatcgtttggatccttcgaataattag

SEQ ID NO: 28 - DNA, 35 bp, synthetic construct
  source 1..35: mol_type = other DNA
gatccaaacgatgcagtttggaaaggttctatttg

SEQ ID NO: 29 - DNA, 30 bp, synthetic construct; identical to SEQ ID NO: 25
  source 1..30: mol_type = other DNA

SEQ ID NO: 30 - DNA, 29 bp, synthetic construct
  source 1..29: mol_type = other DNA
gcacaagcgtgccggaagaagaagaagtg

SEQ ID NO: 31 - DNA, 34 bp, synthetic construct
  source 1..34: mol_type = other DNA
caaactgcatcgtttggatccttcgaataattag

SEQ ID NO: 32 - DNA, 22 bp, synthetic construct
  source 1..22: mol_type = other DNA
gatctaacatccaaagacgaaa

SEQ ID NO: 33 - DNA, 22 bp, synthetic construct
  source 1..22: mol_type = other DNA
ttgagataaatttcacgtttaa

SEQ ID NO: 34 - protein, 710 aa, Homo Sapiens
MKLVFLVLLFLGALGLCLAGRRRSVQWCAVSQPEATKCFQWQRNMRKVRGPPVSCIKRDSPIQCIQAIAENRADAVTLDGGFIYEAGLAPYKLRPVAAEVYGTERQPRTHYYAVAVVKKGGSFQLNELQGLKSCHTGLRRTAGWNVPIGTLRPFLNWTGPPEPIEAAVARFFSASCVPGADKGQFPNLCRLCAGTGENKCAFSSQEPYFSYSGAFKCLRDGAGDVAFIRESTVFEDLSDEAERDEYELLCPDNTRKPVDKFKDCHLARVPSHAVVARSVNGKEDAIWNLLRQAQEKFGKDKSPKFQLFGSPSGQKDLLFKDSAIGFSRVPPRIDSGLYLGSGYFTAIQNLRKSEEEVAARRARVVWCAVGEQELRKCNQWSGLSEGSVTCSSASTTEDCIALVLKGEADAMSLDGGYVYTAGKCGLVPVLAENYKSQQSSDPDPNCVDRPVEGYLAVAVVRRSDTSLTWNSVKGKKSCHTAVDRTAGWNIPMGLLFNQTGSCKFDEYFSQSCAPGSDPRSNLCALCIGDEQGENKCVPNSNERYYGYTGAFRCLAENAGDVAFVKDVTVLQNTDGNNNEAWAKDLKLADFALLCLDGKRKPVTEARSCHLAMAPNHAVVSRMDKVERLKQVLLHQQAKFGRNGSDCPDKFCLFQSETKNLLFNDNTECLARLHGKTTYEKYLGPQYVAGITNLKKCSTSPLLEACEFLRK

SEQ ID NO: 35 - protein, 123 aa, Homo Sapiens
KQFTKCELSQLLKDIDGYGGIALPELICTMFHTSGYDTQAIVENNESTEYGLFQISNKLWCKSSQVPQSRNICDISCDKFLDDDITDDIMCAKKILDIKGIDYWLAHKALCTEKLEQWLCEKL

SEQ ID NO: 36 - protein, 142 aa, Homo Sapiens
MRFFVPLFLVGILFPAILAKQFTKCELSQLLKDIDGYGGIALPELICTMFHTSGYDTQAIVENNESTEYGLFQISNKLWCKSSQVPQSRNICDISCDKFLDDDITDDIMCAKKILDIKGIDYWLAHKALCTEKLEQWLCEKL

SEQ ID NO: 37 - protein, 213 aa, Homo Sapiens
MKFISILFLLIGSVFGAPVNTTTEDETAQIPAEAVIGYSDLEGDFDVAVLPFSNSTNNGLLFINTTIASIAAKEEGVSLEKREAEAYVEFKQFTKCELSQLLKDIDGYGGIALPELICTMFHTSGYDTQAIVENNESTEYGLFQISNKLWCKSSQVPQSRNICDISCDKFLDDDITDDIMCAKKILDIKGIDYWLAHKALCTEKLEQWLCEKL

SEQ ID NO: 38 - protein, 216 aa, Homo Sapiens
MQFGKVLFAISALAVTALGAPVNTTTEDETAQIPAEAVIGYSDLEGDFDVAVLPFSNSTNNGLLFINTTIASIAAKEEGVSLEKREAEAYVEFKQFTKCELSQLLKDIDGYGGIALPELICTMFHTSGYDTQAIVENNESTEYGLFQISNKLWCKSSQVPQSRNICDISCDKFLDDDITDDIMCAKKILDIKGIDYWLAHKALCTEKLEQWLCEKL

SEQ ID NO: 39 - protein, 155 aa, Homo Sapiens
MKFISILFLLIGSVFGAPVAPAEEAANHLHKRKQFTKCELSQLLKDIDGYGGIALPELICTMFHTSGYDTQAIVENNESTEYGLFQISNKLWCKSSQVPQSRNICDISCDKFLDDDITDDIMCAKKILDIKGIDYWLAHKALCTEKLEQWLCEKL

SEQ ID NO: 40 - protein, 158 aa, Homo Sapiens
MQFGKVLFAISALAVTALGAPVAPAEEAANHLHKRKQFTKCELSQLLKDIDGYGGIALPELICTMFHTSGYDTQAIVENNESTEYGLFQISNKLWCKSSQVPQSRNICDISCDKFLDDDITDDIMCAKKILDIKGIDYWLAHKALCTEKLEQWLCEKL

SEQ ID NO: 41 - DNA, 270 bp, synthetic construct
  source 1..270: mol_type = other DNA
atgaaattcatctcaattctgttccttttgataggcagtgtatttggtgctccagtcaacactacaacagaagatgaaacggcacaaattccggctgaagctgtcatcggttactcagatttagaaggggatttcgatgttgctgttttgccattttccaacagcacaaataacgggttattgtttataaatactactattgccagcattgctgctaaagaagaaggggtatctctcgagaaaagagaggctgaagcttatgtcgagttc

SEQ ID NO: 42 - DNA, 279 bp, synthetic construct
  source 1..279: mol_type = other DNA
atgcagtttggaaaggttctatttgctatttctgccctggctgtcacagctctgggagctccagtcaacactacaacagaagatgaaacggcacaaattccggctgaagctgtcatcggttactcagatttagaaggggatttcgatgttgctgttttgccattttccaacagcacaaataacgggttattgtttataaatactactattgccagcattgctgctaaagaagaaggggtatctctcgagaaaagagaggctgaagcttatgtcgagttc

SEQ ID NO: 43 - DNA, 96 bp, synthetic construct
  source 1..96: mol_type = other DNA
atgaaattcatctcaattctgttccttttgataggcagtgtatttggtgctccagttgctccagccgaagaggcagcaaaccacttgcacaagcgt

SEQ ID NO: 44 - DNA, 105 bp, synthetic construct
  source 1..105: mol_type = other DNA
atgcagtttggaaaggttctatttgctatttctgccctggctgtcacagctctgggagctccagttgctccagccgaagaggcagcaaaccacttgcacaagcgt

SEQ ID NO: 45 - DNA, 2079 bp, synthetic construct
  source 1..2079: mol_type = other DNA
gccggaagaagaagaagtgttcaatggtgcgccgttagtcaacctgaggctacaaagtgttttcaatggcagagaaatatgagaaaggttagaggtccacctgtttcttgtatcaagagagattctccaatccaatgtattcaagctattgctgagaacagagctgatgctgttactttggatggtggttttatctacgaagctggtttggctccatataaacttagaccagttgctgctgaggtttacggtactgaaagacaacctagaactcattactatgctgttgctgttgttaagaaaggtggttctttccaattgaacgaattgcaaggtttgaagtcttgtcacactggtttgagaagaactgctggttggaatgttccaattggtactttaagaccatttcttaactggactggtccacctgagccaattgaagctgctgttgctagatttttctctgcttcttgtgttccaggtgctgataagggtcaatttcctaatttgtgtagattgtgtgctggtactggagagaacaaatgtgctttctcttctcaagaaccttacttttcttattctggtgctttcaagtgtttgagagatggtgctggagatgttgcttttattagagagtctactgttttcgaagatttgtctgatgaggctgaaagagatgagtatgaattgttgtgtccagataacactagaaagcctgttgataagtttaaagattgtcatttggctagagttccatctcacgctgttgttgctagatctgttaatggtaaagaggatgctatttggaacttgttgagacaagctcaagaaaagttcggtaaagacaagtctccaaagttccaattgttcggttctccttctggtcaaaaggatttgttgtttaaagattctgctatcggtttctctagagttccacctagaattgattctggtttgtacttgggttctggttacttcactgctatccaaaatttgagaaagtctgaagaggaagttgctgctagaagagctagagttgtttggtgtgctgttggagagcaagaattgagaaagtgtaaccaatggtctggtttgtctgaaggttctgttacttgttcttctgcttctactactgaggattgtattgctttggttttgaaaggtgaagctgatgctatgtctttggatggtggttacgtttatactgctggtaaatgtggtttggttccagttttggctgagaattacaaatctcaacaatcttctgatccagatcctaactgtgttgatagacctgttgaaggttatttggctgttgctgttgttagaagatctgatacttctttgacttggaactctgttaaaggtaaaaagtcttgtcatactgctgttgatagaaccgccggttggaatattccaatgggtttgttgtttaaccaaactggttcttgtaagtttgatgagtacttctctcaatcttgtgctccaggttctgatcctagatctaatttgtgtgctttgtgtattggagatgagcaaggtgaaaacaaatgtgttcctaattctaacgagagatactatggttatactggtgcttttagatgtttggctgaaaacgccggagatgttgctttcgttaaggatgttactgttttgcaaaacactgatggtaacaataacgaagcttgggctaaggatttgaaattggctgatttcgctttgttgtgtttggatggtaaaagaaaaccagttactgaggctagatcttgtcatttggctatggctcctaaccacgctgttgtttctagaatggataaggttgaaagattgaagcaagttttgttgcatcaacaggctaagtttggtagaaatggttctgattgtcctgataagttttgtttgttccaatctgagactaaaaacttgttgttcaatgataacactgaatgtttggctagattgcacggtaaaactacttacgaaaaatatttgggtcctcaatacgttgctggtattactaacttgaagaaatgctccaccagtccattgcttgaggcttgcgagttccttagaaaataa

SEQ ID NO: 46 - DNA, 2349 bp, synthetic construct
  source 1..2349: mol_type = other DNA
atgaaattcatctcaattctgttccttttgataggcagtgtatttggtgctccagtcaacactacaacagaagatgaaacggcacaaattccggctgaagctgtcatcggttactcagatttagaaggggatttcgatgttgctgttttgccattttccaacagcacaaataacgggttattgtttataaatactactattgccagcattgctgctaaagaagaaggggtatctctcgagaaaagagaggctgaagcttatgtcgagttcgccggaagaagaagaagtgttcaatggtgcgccgttagtcaacctgaggctacaaagtgttttcaatggcagagaaatatgagaaaggttagaggtccacctgtttcttgtatcaagagagattctccaatccaatgtattcaagctattgctgagaacagagctgatgctgttactttggatggtggttttatctacgaagctggtttggctccatataaacttagaccagttgctgctgaggtttacggtactgaaagacaacctagaactcattactatgctgttgctgttgttaagaaaggtggttctttccaattgaacgaattgcaaggtttgaagtcttgtcacactggtttgagaagaactgctggttggaatgttccaattggtactttaagaccatttcttaactggactggtccacctgagccaattgaagctgctgttgctagatttttctctgcttcttgtgttccaggtgctgataagggtcaatttcctaatttgtgtagattgtgtgctggtactggagagaacaaatgtgctttctcttctcaagaaccttacttttcttattctggtgctttcaagtgtttgagagatggtgctggagatgttgcttttattagagagtctactgttttcgaagatttgtctgatgaggctgaaagagatgagtatgaattgttgtgtccagataacactagaaagcctgttgataagtttaaagattgtcatttggctagagttccatctcacgctgttgttgctagatctgttaatggtaaagaggatgctatttggaacttgttgagacaagctcaagaaaagttcggtaaagacaagtctccaaagttccaattgttcggttctccttctggtcaaaaggatttgttgtttaaagattctgctatcggtttctctagagttccacctagaattgattctggtttgtacttgggttctggttacttcactgctatccaaaatttgagaaagtctgaagaggaagttgctgctagaagagctagagttgtttggtgtgctgttggagagcaagaattgagaaagtgtaaccaatggtctggtttgtctgaaggttctgttacttgttcttctgcttctactactgaggattgtattgctttggttttgaaaggtgaagctgatgctatgtctttggatggtggttacgtttatactgctggtaaatgtggtttggttccagttttggctgagaattacaaatctcaacaatcttctgatccagatcctaactgtgttgatagacctgttgaaggttatttggctgttgctgttgttagaagatctgatacttctttgacttggaactctgttaaaggtaaaaagtcttgtcatactgctgttgatagaaccgccggttggaatattccaatgggtttgttgtttaaccaaactggttcttgtaagtttgatgagtacttctctcaatcttgtgctccaggttctgatcctagatctaatttgtgtgctttgtgtattggagatgagcaaggtgaaaacaaatgtgttcctaattctaacgagagatactatggttatactggtgcttttagatgtttggctgaaaacgccggagatgttgctttcgttaaggatgttactgttttgcaaaacactgatggtaacaataacgaagcttgggctaaggatttgaaattggctgatttcgctttgttgtgtttggatggtaaaagaaaaccagttactgaggctagatcttgtcatttggctatggctcctaaccacgctgttgtttctagaatggataaggttgaaagattgaagcaagttttgttgcatcaacaggctaagtttggtagaaatggttctgattgtcctgataagttttgtttgttccaatctgagactaaaaacttgttgttcaatgataacactgaatgtttggctagattgcacggtaaaactacttacgaaaaatatttgggtcctcaatacgttgctggtattactaacttgaagaaatgctccaccagtccattgcttgaggcttgcgagttccttagaaaataa

SEQ ID NO: 47 - DNA, 2358 bp, synthetic construct
  source 1..2358: mol_type = other DNA
atgcagtttggaaaggttctatttgctatttctgccctggctgtcacagctctgggagctccagtcaacactacaacagaagatgaaacggcacaaattccggctgaagctgtcatcggttactcagatttagaaggggatttcgatgttgctgttttgccattttccaacagcacaaataacgggttattgtttataaatactactattgccagcattgctgctaaagaagaaggggtatctctcgagaaaagagaggctgaagcttatgtcgagttcgccggaagaagaagaagtgttcaatggtgcgccgttagtcaacctgaggctacaaagtgttttcaatggcagagaaatatgagaaaggttagaggtccacctgtttcttgtatcaagagagattctccaatccaatgtattcaagctattgctgagaacagagctgatgctgttactttggatggtggttttatctacgaagctggtttggctccatataaacttagaccagttgctgctgaggtttacggtactgaaagacaacctagaactcattactatgctgttgctgttgttaagaaaggtggttctttccaattgaacgaattgcaaggtttgaagtcttgtcacactggtttgagaagaactgctggttggaatgttccaattggtactttaagaccatttcttaactggactggtccacctgagccaattgaagctgctgttgctagatttttctctgcttcttgtgttccaggtgctgataagggtcaatttcctaatttgtgtagattgtgtgctggtactggagagaacaaatgtgctttctcttctcaagaaccttacttttcttattctggtgctttcaagtgtttgagagatggtgctggagatgttgcttttattagagagtctactgttttcgaagatttgtctgatgaggctgaaagagatgagtatgaattgttgtgtccagataacactagaaagcctgttgataagtttaaagattgtcatttggctagagttccatctcacgctgttgttgctagatctgttaatggtaaagaggatgctatttggaacttgttgagacaagctcaagaaaagttcggtaaagacaagtctccaaagttccaattgttcggttctccttctggtcaaaaggatttgttgtttaaagattctgctatcggtttctctagagttccacctagaattgattctggtttgtacttgggttctggttacttcactgctatccaaaatttgagaaagtctgaagaggaagttgctgctagaagagctagagttgtttggtgtgctgttggagagcaagaattgagaaagtgtaaccaatggtctggtttgtctgaaggttctgttacttgttcttctgcttctactactgaggattgtattgctttggttttgaaaggtgaagctgatgctatgtctttggatggtggttacgtttatactgctggtaaatgtggtttggttccagttttggctgagaattacaaatctcaacaatcttctgatccagatcctaactgtgttgatagacctgttgaaggttatttggctgttgctgttgttagaagatctgatacttctttgacttggaactctgttaaaggtaaaaagtcttgtcatactgctgttgatagaaccgccggttggaatattccaatgggtttgttgtttaaccaaactggttcttgtaagtttgatgagtacttctctcaatcttgtgctccaggttctgatcctagatctaatttgtgtgctttgtgtattggagatgagcaaggtgaaaacaaatgtgttcctaattctaacgagagatactatggttatactggtgcttttagatgtttggctgaaaacgccggagatgttgctttcgttaaggatgttactgttttgcaaaacactgatggtaacaataacgaagcttgggctaaggatttgaaattggctgatttcgctttgttgtgtttggatggtaaaagaaaaccagttactgaggctagatcttgtcatttggctatggctcctaaccacgctgttgtttctagaatggataaggttgaaagattgaagcaagttttgttgcatcaacaggctaagtttggtagaaatggttctgattgtcctgataagttttgtttgttccaatctgagactaaaaacttgttgttcaatgataacactgaatgtttggctagattgcacggtaaaactacttacgaaaaatatttgggtcctcaatacgttgctggtattactaacttgaagaaatgctccaccagtccattgcttgaggcttgcgagttccttagaaaataa

SEQ ID NO: 48 - DNA, 2175 bp, synthetic construct
  source 1..2175: mol_type = other DNA
atgaaattcatctcaattctgttccttttgataggcagtgtatttggtgctccagttgctccagccgaagaggcagcaaaccacttgcacaagcgtgccggaagaagaagaagtgttcaatggtgcgccgttagtcaacctgaggctacaaagtgttttcaatggcagagaaatatgagaaaggttagaggtccacctgtttcttgtatcaagagagattctccaatccaatgtattcaagctattgctgagaacagagctgatgctgttactttggatggtggttttatctacgaagctggtttggctccatataaacttagaccagttgctgctgaggtttacggtactgaaagacaacctagaactcattactatgctgttgctgttgttaagaaaggtggttctttccaattgaacgaattgcaaggtttgaagtcttgtcacactggtttgagaagaactgctggttggaatgttccaattggtactttaagaccatttcttaactggactggtccacctgagccaattgaagctgctgttgctagatttttctctgcttcttgtgttccaggtgctgataagggtcaatttcctaatttgtgtagattgtgtgctggtactggagagaacaaatgtgctttctcttctcaagaaccttacttttcttattctggtgctttcaagtgtttgagagatggtgctggagatgttgcttttattagagagtctactgttttcgaagatttgtctgatgaggctgaaagagatgagtatgaattgttgtgtccagataacactagaaagcctgttgataagtttaaagattgtcatttggctagagttccatctcacgctgttgttgctagatctgttaatggtaaagaggatgctatttggaacttgttgagacaagctcaagaaaagttcggtaaagacaagtctccaaagttccaattgttcggttctccttctggtcaaaaggatttgttgtttaaagattctgctatcggtttctctagagttccacctagaattgattctggtttgtacttgggttctggttacttcactgctatccaaaatttgagaaagtctgaagaggaagttgctgctagaagagctagagttgtttggtgtgctgttggagagcaagaattgagaaagtgtaaccaatggtctggtttgtctgaaggttctgttacttgttcttctgcttctactactgaggattgtattgctttggttttgaaaggtgaagctgatgctatgtctttggatggtggttacgtttatactgctggtaaatgtggtttggttccagttttggctgagaattacaaatctcaacaatcttctgatccagatcctaactgtgttgatagacctgttgaaggttatttggctgttgctgttgttagaagatctgatacttctttgacttggaactctgttaaaggtaaaaagtcttgtcatactgctgttgatagaaccgccggttggaatattccaatgggtttgttgtttaaccaaactggttcttgtaagtttgatgagtacttctctcaatcttgtgctccaggttctgatcctagatctaatttgtgtgctttgtgtattggagatgagcaaggtgaaaacaaatgtgttcctaattctaacgagagatactatggttatactggtgcttttagatgtttggctgaaaacgccggagatgttgctttcgttaaggatgttactgttttgcaaaacactgatggtaacaataacgaagcttgggctaaggatttgaaattggctgatttcgctttgttgtgtttggatggtaaaagaaaaccagttactgaggctagatcttgtcatttggctatggctcctaaccacgctgttgtttctagaatggataaggttgaaagattgaagcaagttttgttgcatcaacaggctaagtttggtagaaatggttctgattgtcctgataagttttgtttgttccaatctgagactaaaaacttgttgttcaatgataacactgaatgtttggctagattgcacggtaaaactacttacgaaaaatatttgggtcctcaatacgttgctggtattactaacttgaagaaatgctccaccagtccattgcttgaggcttgcgagttccttagaaaataa

SEQ ID NO: 49 - DNA, 2184 bp, synthetic construct
  source 1..2184: mol_type = other DNA
atgcagtttggaaaggttctatttgctatttctgccctggctgtcacagctctgggagctccagttgctccagccgaagaggcagcaaaccacttgcacaagcgtgccggaagaagaagaagtgttcaatggtgcgccgttagtcaacctgaggctacaaagtgttttcaatggcagagaaatatgagaaaggttagaggtccacctgtttcttgtatcaagagagattctccaatccaatgtattcaagctattgctgagaacagagctgatgctgttactttggatggtggttttatctacgaagctggtttggctccatataaacttagaccagttgctgctgaggtttacggtactgaaagacaacctagaactcattactatgctgttgctgttgttaagaaaggtggttctttccaattgaacgaattgcaaggtttgaagtcttgtcacactggtttgagaagaactgctggttggaatgttccaattggtactttaagaccatttcttaactggactggtccacctgagccaattgaagctgctgttgctagatttttctctgcttcttgtgttccaggtgctgataagggtcaatttcctaatttgtgtagattgtgtgctggtactggagagaacaaatgtgctttctcttctcaagaaccttacttttcttattctggtgctttcaagtgtttgagagatggtgctggagatgttgcttttattagagagtctactgttttcgaagatttgtctgatgaggctgaaagagatgagtatgaattgttgtgtccagataacactagaaagcctgttgataagtttaaagattgtcatttggctagagttccatctcacgctgttgttgctagatctgttaatggtaaagaggatgctatttggaacttgttgagacaagctcaagaaaagttcggtaaagacaagtctccaaagttccaattgttcggttctccttctggtcaaaaggatttgttgtttaaagattctgctatcggtttctctagagttccacctagaattgattctggtttgtacttgggttctggttacttcactgctatccaaaatttgagaaagtctgaagaggaagttgctgctagaagagctagagttgtttggtgtgctgttggagagcaagaattgagaaagtgtaaccaatggtctggtttgtctgaaggttctgttacttgttcttctgcttctactactgaggattgtattgctttggttttgaaaggtgaagctgatgctatgtctttggatggtggttacgtttatactgctggtaaatgtggtttggttccagttttggctgagaattacaaatctcaacaatcttctgatccagatcctaactgtgttgatagacctgttgaaggttatttggctgttgctgttgttagaagatctgatacttctttgacttggaactctgttaaaggtaaaaagtcttgtcatactgctgttgatagaaccgccggttggaatattccaatgggtttgttgtttaaccaaactggttcttgtaagtttgatgagtacttctctcaatcttgtgctccaggttctgatcctagatctaatttgtgtgctttgtgtattggagatgagcaaggtgaaaacaaatgtgttcctaattctaacgagagatactatggttatactggtgcttttagatgtttggctgaaaacgccggagatgttgctttcgttaaggatgttactgttttgcaaaacactgatggtaacaataacgaagcttgggctaaggatttgaaattggctgatttcgctttgttgtgtttggatggtaaaagaaaaccagttactgaggctagatcttgtcatttggctatggctcctaaccacgctgttgtttctagaatggataaggttgaaagattgaagcaagttttgttgcatcaacaggctaagtttggtagaaatggttctgattgtcctgataagttttgtttgttccaatctgagactaaaaacttgttgttcaatgataacactgaatgtttggctagattgcacggtaaaactacttacgaaaaatatttgggtcctcaatacgttgctggtattactaacttgaagaaatgctccaccagtccattgcttgaggcttgcgagttccttagaaaataa